European Patent Application EP 4 711 444 A2, published March 18, 2026. Title: ENDOTHELIAL CELLS FOR MITIGATION OF CHEMOTHERAPY-INDUCED TOXICITY. Applicant: Angiocrine Bioscience, Inc. Application EP. The sequence listing filed with the application follows.

SEQUENCE LISTING (1 sequence)

SEQ ID NO: 1 - protein, 128 aa, synthetic construct
MAAAVEALFVVLEREGAILPRQEGFSGVYVFFSPINFVIPPMGAVMLSLRLRVCIPPGYFGRFLALTDVNQPDVFTESYIMTPDMTEELSVVLFNHGDQFFYGHAGMAVVRLMLIRVVFPVVRQASNV